European Patent Specification EP 3 878 868 B1, published October 9, 2024. Title: High Affinity Human Antibodies Against Human Interleukin-4 Receptor alpha and Uses Thereof. Applicant: AJOU UNIVERSITY INDUSTRY-ACADEMIC COOPERATION FOUNDATION. The sequence listing filed with the application follows.

SEQUENCE LISTING (98 sequences)

SEQ ID NO: 1 - protein, 116 aa, Artificial Sequence
  Synthetic Sequence
EVQLLESGGGLVQPGGSLRLSCAVSGFTFSNYAMSWVRQAPGKGLEWVSAISSGGGNIYYADSVKGRFTISRDNSKNTLYLQMNSLRAEDTAVYYCAKLRRYFDYWGQGTLVTVSS

SEQ ID NO: 2 - protein, 121 aa, Artificial Sequence
  Synthetic Sequence
EVQLLESGGGLVQPGGSLRLSCAASGFTFSDYAMSWVRQAPGKGLEWVSAISSGGSSIYYADSVKGRFTISRDNSKNTLHLQMNSLRAEDTAVYYCARGPQRSATAVFDYWGQGTLVTVSS

SEQ ID NO: 3 - protein, 127 aa, Artificial Sequence
  Synthetic Sequence
EVQLLESGGGLVQPGGSLRLSCAASGFTFSNYAMSWVRQAPGKGLEWVSWISPNSGNIYYADSVKGRFTISRDNSKNTLYLQMNSLRAEDTAVYYCARRPLSAAWSHSSYYNAMDVWGQGTLVTVSS

SEQ ID NO: 4 - protein, 116 aa, Artificial Sequence
  Synthetic Sequence
EVQLLESGGGLVQPGGSLRLSCAASGFTFSGYAMSWVRQAPGKGLEWVSLISHSGSNTYYADSVKGRFTISRDNSKNTLYLQMNSLRAEDTAVYYCARPHRAFDYWGQGTLVTVSS

SEQ ID NO: 5 - protein, 116 aa, Artificial Sequence
  Synthetic Sequence
EVQLLESGGGLVQPGGSLRLSCAASGFTFSNYAMSWVRQAPGKGLEWVSGISHGSGSIYYADSVKGRFTISRDNSKNTLYLQMNSLRAEDTAVYYCARPHRAFDYWGQGTLVTVSS

SEQ ID NO: 6 - protein, 116 aa, Artificial Sequence
  Synthetic Sequence
EVQLLESGGGLVQPGGSLRLSCAASGFTFSNYAMSWVRQAPGKGLEWVSGISHGNGSIYYADSVKGRFTISRDNSKNTLYLQMNSLRAEDTAVYYCAKTGRHFDYWGQGTLVTVSS

SEQ ID NO: 7 - protein, 116 aa, Artificial Sequence
  Synthetic Sequence
EVQLLESGGGLVQPGGSLRLSCAASGFTFSNYAMSWVRQAPGKGLEWVSSISPSGSSIYYADSVKGRFTISRDNSKNTLYLQMNSLRAEDTAVYYCARSYRAFDYWGQGTLVTVSS

SEQ ID NO: 8 - protein, 116 aa, Artificial Sequence
  Synthetic Sequence
EVQLLESGGGLVQPGGSLRLSCAASGFTFSNYAMSWVRQAPGKGLEWVSAISPSGGSIYYADSVKGRFTISRDNSKNTLYLQMNSLRAEDTAVYYCARAKRAFDYWGQGTLVTVSS

SEQ ID NO: 9 - protein, 116 aa, Artificial Sequence
  Synthetic Sequence
EVQLLESGGGLVQPGGSLRLSCAASGFTFSNYAMSWVRQAPGKGLEWVSAISPGSGSTYYADSVKGRFTISRDNSKNTLYLQMNSLRAEDTAVYYCAKFRRHFDYWGQGTLVTVSS

SEQ ID NO: 10 - protein, 116 aa, Artificial Sequence
  Synthetic Sequence
EVQLLESGGGLVQPGGSLRLSCAASGFTFSNYAMSWVRQAPGKGLEWVSAISSGGGNIYYADSVKGRFTISRDNSKNTLYLQMNSLRAEDTAVYYCARVHRAFDYWGQGTLVTVSS

SEQ ID NO: 11 - protein, 5 aa, Artificial Sequence
  Synthetic Sequence
NYAMS

SEQ ID NO: 12 - protein, 5 aa, Artificial Sequence
  Synthetic Sequence
DYAMS

SEQ ID NO: 13 - protein, 5 aa, Artificial Sequence
  Synthetic Sequence
GYAMS

SEQ ID NO: 14 - protein, 17 aa, Artificial Sequence
  Synthetic Sequence
AISSGGGNIYYADSVKG

SEQ ID NO: 15 - protein, 17 aa, Artificial Sequence
  Synthetic Sequence
AISSGGSSIYYADSVKG

SEQ ID NO: 16 - protein, 17 aa, Artificial Sequence
  Synthetic Sequence
WISPNSGNIYYADSVKG

SEQ ID NO: 17 - protein, 17 aa, Artificial Sequence
  Synthetic Sequence
LISHSGSNTYYADSVKG

SEQ ID NO: 18 - protein, 17 aa, Artificial Sequence
  Synthetic Sequence
GISHGSGSIYYADSVKG

SEQ ID NO: 19 - protein, 17 aa, Artificial Sequence
  Synthetic Sequence
GISHGNGSIYYADSVKG

SEQ ID NO: 20 - protein, 17 aa, Artificial Sequence
  Synthetic Sequence
SISPSGSSIYYADSVKG

SEQ ID NO: 21 - protein, 17 aa, Artificial Sequence
  Synthetic Sequence
AISPSGGSIYYADSVKG

SEQ ID NO: 22 - protein, 17 aa, Artificial Sequence
  Synthetic Sequence
AISPGSGSTYYADSVKG

SEQ ID NO: 23 - protein, 7 aa, Artificial Sequence
  Synthetic Sequence
LRRYFDY

SEQ ID NO: 24 - protein, 12 aa, Artificial Sequence
  Synthetic Sequence
GPQRSATAVFDY

SEQ ID NO: 25 - protein, 18 aa, Artificial Sequence
  Synthetic Sequence
RPLSAAWSHSSYYNAMDV

SEQ ID NO: 26 - protein, 7 aa, Artificial Sequence
  Synthetic Sequence
PHRAFDY

SEQ ID NO: 27 - protein, 7 aa, Artificial Sequence
  Synthetic Sequence
TGRDFDY

SEQ ID NO: 28 - protein, 7 aa, Artificial Sequence
  Synthetic Sequence
TGRHFDY

SEQ ID NO: 29 - protein, 7 aa, Artificial Sequence
  Synthetic Sequence
SYRAFDY

SEQ ID NO: 30 - protein, 7 aa, Artificial Sequence
  Synthetic Sequence
AKRAFDY

SEQ ID NO: 31 - protein, 7 aa, Artificial Sequence
  Synthetic Sequence
FRRHFDY

SEQ ID NO: 32 - protein, 7 aa, Artificial Sequence
  Synthetic Sequence
VHRAFDY

SEQ ID NO: 33 - protein, 110 aa, Artificial Sequence
  Synthetic Sequence
QSVLTQPPSASGTPGQRVTISCSGSSSNIGNNYVNWYQQLPGTAPKLLIYDNSHRPSGVPDRFSGSKSGTSASLAISGLRSEDEADYYCGTWDASLSAYVFGGGTKLTVL

SEQ ID NO: 34 - protein, 110 aa, Artificial Sequence
  Synthetic Sequence
QSVLTQPPSASGTPGQRVTISCSGSSSNIGNNNVSWYQQLPGTAPKLLIYANSKRPSGVPDRFSGSKSGTSASLAISGLRSEDEADYYCGSWDDSLSAYVFGGGTKLTVL

SEQ ID NO: 35 - protein, 110 aa, Artificial Sequence
  Synthetic Sequence
QSVLTQPPSAPGTPGQRVTISCTGSSSNIGSNSVNWYQQLPGTAPKLLIYDDSHRPSGVPDRFSGSKSGTSASLAISGLRSEDEADYYCDAWDSSLSAYVFGGGTKLTVL

SEQ ID NO: 36 - protein, 110 aa, Artificial Sequence
  Synthetic Sequence
QSVLTQPPSASGTPGQRVTLSCTGSSSNIGSNYVSWYQQLPGTAPKLLIYADSQRPSGVPDRFSGSKSGTSASLAISGLRSEDEADYYCGTWDDSLSGYVFGGGTKLTVL

SEQ ID NO: 37 - protein, 110 aa, Artificial Sequence
  Synthetic Sequence
QSVLTQPPSASGTPGQRVTISCSSSSSNIGSNYVSWYQQLPGTAPKLLIYSDSHRPSGVPDRFSGSKSGTSASLAISGLRSEDEADYYCGSWDYSLSAYVFGGGTKLTVL

SEQ ID NO: 38 - protein, 110 aa, Artificial Sequence
  Synthetic Sequence
QSVLTQPPSASGTPGQRVTISCTGSSSNIGNNTVSWYQQLPGTAPKLLIYDNSHRPSGVPDRFSGSKSGTSASLAISGLQSEDEADYYCGSWDYSLSAYVFGGGTKLTVL

SEQ ID NO: 39 - protein, 110 aa, Artificial Sequence
  Synthetic Sequence
QSVLTQPPSASGTPGQRVTISCTGSSSNIGNNDVNWYQQLPGTAPKLLIYYDSQRPSGVPDRFSGSKSGTSASLAISGLRSEDEADYYCATWDASLSAYVFGGGTKLTVL

SEQ ID NO: 40 - protein, 110 aa, Artificial Sequence
  Synthetic Sequence
QSVLTQPPSASGTPGQRVTISCSGSSSNIGSNAVNWYQQLPGTAPKLLIYYDNQRPSGVPDRFSGSKSGTSASLAISGLRSEDEADYYCGTWDDSLNGYVFGGGTKLTVL

SEQ ID NO: 41 - protein, 110 aa, Artificial Sequence
  Synthetic Sequence
QSVLTQPPSASGTPGQRVTISCSGSSSNIGNNAVTWYQQLPGTAPKLLIYDDSHRPSGVPDRFSGSKSGTSASLAISGLRSEDEADYYCGSWDYSLSAYVFGGGTKLTVL

SEQ ID NO: 42 - protein, 110 aa, Artificial Sequence
  Synthetic Sequence
QSVLTQPPSASGTPGQRVTISCSGSSSNIGSNTFNWYQQLPGTAPKLLIYADSHRPSGVPDRFSGSKSGTSASLAISGLRSEDEADYYCGTWDYSLSGYVLGGGTKLTVL

SEQ ID NO: 43 - protein, 13 aa, Artificial Sequence
  Synthetic Sequence
SGSSSNIGNNYVN

SEQ ID NO: 44 - protein, 13 aa, Artificial Sequence
  Synthetic Sequence
SGSSSNIGNNNVS

SEQ ID NO: 45 - protein, 13 aa, Artificial Sequence
  Synthetic Sequence
TGSSSNIGSNSVN

SEQ ID NO: 46 - protein, 13 aa, Artificial Sequence
  Synthetic Sequence
TGSSSNIGSNYVS

SEQ ID NO: 47 - protein, 13 aa, Artificial Sequence
  Synthetic Sequence
SSSSSNIGSNYVS

SEQ ID NO: 48 - protein, 13 aa, Artificial Sequence
  Synthetic Sequence
TGSSSNIGNNTVS

SEQ ID NO: 49 - protein, 13 aa, Artificial Sequence
  Synthetic Sequence
TGSSSNIGNNDVN

SEQ ID NO: 50 - protein, 13 aa, Artificial Sequence
  Synthetic Sequence
SGSSSNIGSNAVN

SEQ ID NO: 51 - protein, 13 aa, Artificial Sequence
  Synthetic Sequence
SGSSSNIGNNAVT

SEQ ID NO: 52 - protein, 13 aa, Artificial Sequence
  Synthetic Sequence
SGSSSNIGSNTFN

SEQ ID NO: 53 - protein, 7 aa, Artificial Sequence
  Synthetic Sequence
DNSHRPS

SEQ ID NO: 54 - protein, 7 aa, Artificial Sequence
  Synthetic Sequence
ANSKRPS

SEQ ID NO: 55 - protein, 7 aa, Artificial Sequence
  Synthetic Sequence
DDSHRPS

SEQ ID NO: 56 - protein, 7 aa, Artificial Sequence
  Synthetic Sequence
ADSQRPS

SEQ ID NO: 57 - protein, 7 aa, Artificial Sequence
  Synthetic Sequence
SDSHRPS

SEQ ID NO: 58 - protein, 7 aa, Artificial Sequence
  Synthetic Sequence
YDSQRPS

SEQ ID NO: 59 - protein, 7 aa, Artificial Sequence
  Synthetic Sequence
YDNQRPS

SEQ ID NO: 60 - protein, 7 aa, Artificial Sequence
  Synthetic Sequence
ADSHRPS

SEQ ID NO: 61 - protein, 11 aa, Artificial Sequence
  Synthetic Sequence
GTWDASLSAYV

SEQ ID NO: 62 - protein, 11 aa, Artificial Sequence
  Synthetic Sequence
GSWDDSLSAYV

SEQ ID NO: 63 - protein, 11 aa, Artificial Sequence
  Synthetic Sequence
DAWDSSLSAYV

SEQ ID NO: 64 - protein, 11 aa, Artificial Sequence
  Synthetic Sequence
GTWDDSLSGYV

SEQ ID NO: 65 - protein, 11 aa, Artificial Sequence
  Synthetic Sequence
GSWDYSLSAYV

SEQ ID NO: 66 - protein, 11 aa, Artificial Sequence
  Synthetic Sequence
ATWDASLSAYV

SEQ ID NO: 67 - protein, 11 aa, Artificial Sequence
  Synthetic Sequence
GTWDDSLNGYV

SEQ ID NO: 68 - protein, 11 aa, Artificial Sequence
  Synthetic Sequence
GTWDYSLSGYV

SEQ ID NO: 69 - protein, 116 aa, Artificial Sequence
  Synthetic Sequence
EVQLLESGGGLVQPGGSLRLSCAASGFTFSNYAMSWVRQAPGKGLEWVSAITSSGRSIYYADSVKGRFTISRDNSKNTLYLQMNSLRAEDTAVYYCARVHRAFDYWGQGTLVTVSS

SEQ ID NO: 70 - protein, 116 aa, Artificial Sequence
  Synthetic Sequence
EVQLLESGGGLVQPGGSLRLSCAASGFTFSNYAMSWVRQAPGKGLEWVSAITSSGANIYYADSVKGRFTISRDNSKNTLYLQMNSLRAEDTAVYYCARVHRAFDYWGQGTLVTVSS

SEQ ID NO: 71 - protein, 116 aa, Artificial Sequence
  Synthetic Sequence
EVQLLESGGGLVQPGGSLRLSCAASGFTFSNYAMSWVRQAPGKGLEWVSAITSSGGNIYYADSVKGRFTISRDNSKNTLYLQMNSLRAEDTAVYYCARVHRAFDYWGQGTLVTVSS

SEQ ID NO: 72 - protein, 116 aa, Artificial Sequence
  Synthetic Sequence
EVQLLESGGGLVQPGGSLRLSCAASGFTFSNYAMSWVRQAPGKGLEWVSAITAGGGSIYYADSVKGRFTISRDNSKNTLYLQMNSLRAEDTAVYYCARVHRAFDYWGQGTLVTVSS

SEQ ID NO: 73 - protein, 17 aa, Artificial Sequence
  Synthetic Sequence
AITSSGRSIYYADSVKG

SEQ ID NO: 74 - protein, 17 aa, Artificial Sequence
  Synthetic Sequence
AITSSGANIYYADSVKG

SEQ ID NO: 75 - protein, 17 aa, Artificial Sequence
  Synthetic Sequence
AITSSGGNIYYADSVKG

SEQ ID NO: 76 - protein, 17 aa, Artificial Sequence
  Synthetic Sequence
AITAGGGSIYYADSVKG

SEQ ID NO: 77 - protein, 110 aa, Artificial Sequence; identical to SEQ ID NO: 42
  Synthetic Sequence

SEQ ID NO: 78 - protein, 110 aa, Artificial Sequence
  Synthetic Sequence
QSVLTQPPSASGTPGQRVTISCSGSSSNIGSNTFNWYQQLPGTAPKLLIYADSHRPSGVPDRFSGSKSGTSASLAISGLRSEDEADYYCGTWDYSLRGYVLGGGTKLTVL

SEQ ID NO: 79 - protein, 110 aa, Artificial Sequence
  Synthetic Sequence
QSVLTQPPSASGTPGQRVTISCSGSSSNIGSNTFNWYQQLPGTAPKLLIYADSHRPSGVPDRFSGSKSGTSASLAISGLRSEDEADYYCGYWDYSLSGYVLGGGTKLTVL

SEQ ID NO: 80 - protein, 110 aa, Artificial Sequence; identical to SEQ ID NO: 42
  Synthetic Sequence

SEQ ID NO: 81 - protein, 11 aa, Artificial Sequence
  Synthetic Sequence
GTWDYSLRGYV

SEQ ID NO: 82 - protein, 11 aa, Artificial Sequence
  Synthetic Sequence
GYWDYSLSGYV

SEQ ID NO: 83 - protein, 116 aa, Artificial Sequence
  Synthetic Sequence
EVQLLESGGGLVQPGGSLRLSCAASGFTFSRHAMAWVRQAPGKGLEWVSAITSSGRSIYYADSVKGRFTISRDNSKNTLYLQMNSLRAEDTAVYYCARVHRAFDYWGQGTLVTVSS

SEQ ID NO: 84 - protein, 5 aa, Artificial Sequence
  Synthetic Sequence
RHAMA

SEQ ID NO: 85 - protein, 17 aa, Artificial Sequence
  Synthetic Sequence
AITSSGRSIYYADSVKG

SEQ ID NO: 86 - protein, 111 aa, Artificial Sequence
  Synthetic Sequence
QSVLTQPPSASGTPGQRVTISCSGSSANSRTDGFNWYQQLPGTAPKLLIYADSHRPSGVPDRFSGSKSGTSASLAISGLRSEDEADYYCGTWDYSLSGYVLGGGTKLTVLG

SEQ ID NO: 87 - protein, 111 aa, Artificial Sequence
  Synthetic Sequence
QSVLTQPPSASGTPGQRVTISCSGSAQFGSRDNFNWYQQLPGTAPKLLIYADSHRPSGVPDRFSGSKSGTSASLAISGLRSEDEADYYCGTWDYSLSGYVLGGGTKLTVLG

SEQ ID NO: 88 - protein, 111 aa, Artificial Sequence
  Synthetic Sequence
QSVLTQPPSASGTPGQRVTISCSGSTKQMHNYQFNWYQQLPGTAPKLLIYADSHRPSGVPDRFSGSKSGTSASLAISGLRSEDEADYYCGTWDYSLSGYVLGGGTKLTVLG

SEQ ID NO: 89 - protein, 111 aa, Artificial Sequence
  Synthetic Sequence
QSVLTQPPSASGTPGQRVTISCSGSLLRGENLQFNWYQQLPGTAPKLLIYADSHRPSGVPDRFSGSKSGTSASLAISGLRSEDEADYYCGTWDYSLSGYVLGGGTKLTVLG

SEQ ID NO: 90 - protein, 111 aa, Artificial Sequence
  Synthetic Sequence
QSVLTQPPSASGTPGQRVTISCSGSPLFPDSGSFNWYQQLPGTAPKLLIYADSHRPSGVPDRFSGSKSGTSASLAISGLRSEDEADYYCGTWDYSLSGYVLGGGTKLTVLG

SEQ ID NO: 91 - protein, 111 aa, Artificial Sequence
  Synthetic Sequence
QSVLTQPPSASGTPGQRVTISCSGSAALDLSPSFNWYQQLPGTAPKLLIYADSHRPSGVPDRFSGSKSGTSASLAISGLRSEDEADYYCGTWDYSLSGYVLGGGTKLTVLG

SEQ ID NO: 92 - protein, 13 aa, Artificial Sequence
  Synthetic Sequence
SGSSANSRTDGFN

SEQ ID NO: 93 - protein, 13 aa, Artificial Sequence
  Synthetic Sequence
SGSAQFGSRDNFN

SEQ ID NO: 94 - protein, 13 aa, Artificial Sequence
  Synthetic Sequence
SGSTKQMHNYQFN

SEQ ID NO: 95 - protein, 13 aa, Artificial Sequence
  Synthetic Sequence
SGSLLRGENLQFN

SEQ ID NO: 96 - protein, 13 aa, Artificial Sequence
  Synthetic Sequence
SGSPLFPDSGSFN

SEQ ID NO: 97 - protein, 13 aa, Artificial Sequence
  Synthetic Sequence
SGSAALDLSPSFN

SEQ ID NO: 98 - protein, 232 aa, Artificial Sequence
  Synthetic Sequence
MGWLCSGLLFPVSCLVLLQVASSGNMKVLQEPTCVSDYMSISTCEWKMNGPTNCSTELRLLYQLVFLLSEAHTCIPENNGGAGCVCHLLMDDVVSADNYTLDLWAGQQLLWKGSFKPSEHVKPRAPGNLTVHTNVSDTLLLTWSNPYPPDNYLYNHLTYAVNIWSENDPADFRIYNVTYLEPSLRIAASTLKSGISYRARVRAWAQCYNTTWSEWSPSTKWHNSYREPFEQH